European Patent Specification EP 3 479 840 B1, published September 23, 2026. Title: A method for suppressing decrease in renal functions in non-human animals. Applicant: Kaneka Corporation. The sequence listing filed with the application follows.

SEQUENCE LISTING (3 sequences)

SEQ ID NO: 1 - DNA, 579 bp, Felis catus
atggggtcgtgcgaatgtcctgccctgctgcttctgctatctttgctgctgcttcccctgggcctcccagtcctgggcgccccccctcgcctcatctgtgacagccgagtcctggagaggtacattctggaggccagggaggccgaaaatgtcacgatgggctgtgctgaaggctgcagcttcagtgagaatatcactgtcccagacaccaaggtcaacttctatacctggaagaggatggacgtcgggcagcaggctgtggaagtctggcagggcctcgccctgctctcagaagccatcctgcggggccaggccctgctggccaactcctcccagccatctgagaccctgcagctgcatgtggataaagccgtcagcagcctgcgcagcctcacctccctgcttcgggcactgggagcccggaaggaagccacctcccttccagaggcaacctctgctgctccactccgaacattcactgtcgatactttgtgcaaacttttccgaatctactccaacttcctgcggggaaagctgacgctgtacacaggggaggcctgccgaagaggagacaggtga

SEQ ID NO: 2 - protein, 192 aa, Felis catus
MGSCECPALLLLLSLLLLPLGLPVLGAPPRLICDSRVLERYILEAREAENVTMGCAEGCSFSENITVPDTKVNFYTWKRMDVGQQAVEVWQGLALLSEAILRGQALLANSSQPSETLQLHVDKAVSSLRSLTSLLRALGARKEATSLPEATSAAPLRTFTVDTLCKLFRIYSNFLRGKLTLYTGEACRRGDR

SEQ ID NO: 3 - protein, 165 aa, Felis catus
APPRLICDSRVLERYILEAREAENVTMGCAEGCSFSENITVPDTKVNFYTWKRMDVGQQAVEVWQGLALLSEAILRGQALLANSSQPSETLQLHVDKAVSSLRSLTSLLRALGARKEATSLPEATSAAPLRTFTVDTLCKLFRIYSNFLRGKLTLYTGEACRRGD